European Patent Application EP 4 198 123 A1, published June 21, 2023. Title: Besonders geeignete 3-Desoxyarabinoheptulosanat-7-phosphat-Synthase zur fermentativen Herstellung von ortho-Aminobenzoesäure. Applicant: Covestro Deutschland AG. The sequence listing filed with the application follows.

SEQUENCE LISTING (18 sequences)

SEQ ID NO: 1 - DNA, 1070 bp, artificial sequence
  Expressionskonstrukt
gccctgcaggtaaaaaaaggattgtgacttctccagcaacactgaaagttctcaacgcctacttggataaccccactccaaccctggaggaggcaattgaggtgttcaccccgctgaccgtgggtgaatacgatgacgtgcacatcgcagcgctgcttgccaccatccgtactcgcggtgagcagttcgctgatattgccggcgctgccaaggcgttcctcgcggcggctcgtccgttcccgattactggcgcaggtttgctagattccgctggtactggtggcgacggtgccaacaccatcaacatcaccaccggcgcatccctgatcgcagcatccggtggagtgaagctggttaagcacggcaaccgttcggtgagctccaagtccggctccgccgatgtgctggaagcgctgaatattcctttgggccttgatgtggatcgtgctgtgaagtggttcgaagcgtccaacttcaccttcctgttcgcacctgcgtacaaccctgcgattgcgcatgtgcagccggttcgccaggcgctgaaattccccaccatcttcaacacgcttggaccattgctgtccccggcgcgcccggagcgtcagatcatgggcgtggccaatgccaatcatggacagctcatcgccgaggtcttccgcgagttgggccgtacacgcgcgcttgttgtgcatggcgcaggcaccgatgagatcgcagtccacggcaccaccttggtgtgggagcttaaagaagacggcaccatcgagcattacaccatcgagcctgaggaccttggccttggccgctacacccttgaggatctcgtaggtggcctcggcactgagaacgccgaagctatgcgcgctactttcgcgggcaccggccctgatgcacaccgtgatgcgttggctgcgtccgcaggtgcgatgttctacctcaacggcgatgtcgactccttgaaagatggtgcacaaaaggcgctttccttgcttgccgacggcaccacccaggcatggttggccaagcacgaagagatcgattactcagaaaaggagtcttccaatgactag

SEQ ID NO: 2 - DNA, 1070 bp, artificial sequence
  Expressionskonstrukt
gccctgcaggtaaaaaaaggattttgacttctccagcaacactgaaagttctcaacgcctacttggataaccccactccaaccctggaggaggcaattgaggtgttcaccccgctgaccgtgggtgaatacgatgacgtgcacatcgcagcgctgcttgccaccatccgtactcgcggtgagcagttcgctgatattgccggcgctgccaaggcgttcctcgcggcggctcgtccgttcccgattactggcgcaggtttgctagattccgctggtactggtggcgacggtgccaacaccatcaacatcaccaccggcgcatccctgatcgcagcatccggtggagtgaagctggttaagcacggcaaccgttcggtgagctccaagtccggctccgccgatgtgctggaagcgctgaatattcctttgggccttgatgtggatcgtgctgtgaagtggttcgaagcgtccaacttcaccttcctgttcgcacctgcgtacaaccctgcgattgcgcatgtgcagccggttcgccaggcgctgaaattccccaccatcttcaacacgcttggaccattgctgtccccggcgcgcccggagcgtcagatcatgggcgtggccaatgccaatcatggacagctcatcgccgaggtcttccgcgagttgggccgtacacgcgcgcttgttgtgcatggcgcaggcaccgatgagatcgcagtccacggcaccaccttggtgtgggagcttaaagaagacggcaccatcgagcattacaccatcgagcctgaggaccttggccttggccgctacacccttgaggatctcgtaggtggcctcggcactgagaacgccgaagctatgcgcgctactttcgcgggcaccggccctgatgcacaccgtgatgcgttggctgcgtccgcaggtgcgatgttctacctcaacggcgatgtcgactccttgaaagatggtgcacaaaaggcgctttccttgcttgccgacggcaccacccaggcatggttggccaagcacgaagagatcgattactcagaaaaggagtcttccaatgactag

SEQ ID NO: 3 - protein, 348 aa, Corynebacterium glutamicum
MTSPATLKVLNAYLDNPTPTLEEAIEVFTPLTVGEYDDVHIAALLATIRTRGEQFADIAGAAKAFLAAARPFPITGAGLLDSAGTGGDGANTINITTGASLIAASGGVKLVKHGNRSVSSKSGSADVLEALNIPLGLDVDRAVKWFEASNFTFLFAPAYNPAIAHVQPVRQALKFPTIFNTLGPLLSPARPERQIMGVANANHGQLIAEVFRELGRTRALVVHGAGTDEIAVHGTTLVWELKEDGTIEHYTIEPEDLGLGRYTLEDLVGGLGTENAEAMRATFAGTGPDAHRDALAASAGAMFYLNGDVDSLKDGAQKALSLLADGTTQAWLAKHEEIDYSEKESSND

SEQ ID NO: 4 - protein, 919 aa, Corynebacterium glutamicum
MTDFLRDDIRFLGQILGEVIAEQEGQEVYELVEQARLTSFDIAKGNAEMDSLVQVFDGITPAKATPIARAFSHFALLANLAEDLYDEELREQALDAGDTPPDSTLDATWLKLNEGNVGAEAVADVLRNAEVAPVLTAHPTETRRRTVFDAQKWITTHMRERHALQSAEPTARTQSKLDEIEKNIRRRITILWQTALIRVARPRIEDEIEVGLRYYKLSLLEEIPRINRDVAVELRERFGEGVPLKPVVKPGSWIGGDHDGNPYVTAETVEYSTHRAAETVLKYYARQLHSLEHELSLSDRMNKVTPQLLALADAGHNDVPSRVDEPYRRAVHGVRGRILATTAELIGEDAVEGVWFKVFTPYASPEEFLNDALTIDHSLRESKDVLIADDRLSVLISAIESFGFNLYALDLRQNSESYEDVLTELFERAQVTANYRELSEAEKLEVLLKELRSPRPLIPHGSDEYSEVTDRELGIFRTASEAVKKFGPRMVPHCIISMASSVTDVLEPMVLLKEFGLIAANGDNPRGTVDVIPLFETIEDLQAGAGILDELWKIDLYRNYLLQRDNVQEVMLGYSDSNKDGGYFSANWALYDAELQLVELCRSAGVKLRLFHGRGGTVGRGGGPSYDAILAQPRGAVQGSVRITEQGEIISAKYGNPETARRNLEALVSATLEASLLDVSELTDHQRAYDIMSEISELSLKKYASLVHEDQGFIDYFTQSTPLQEIGSLNIGSRPSSRKQTSSVEDLRAIPWVLSWSQSRVMLPGWFGVGTALEQWIGEGEQATQRIAELQTLNESWPFFTSVLDNMAQVMSKAELRLAKLYADLIPDTEVAERVYSVIREEYFLTKKMFCVITGSDDLLDDNPLLARSVQRRYPYLLPLNVIQVEMMRRYRKGDQSEQVSRNIQLTMNGLSTALRNSG

SEQ ID NO: 5 - DNA, 2760 bp, Corynebacterium glutamicum
atgactgattttttacgcgatgacatcaggttcctcggtcaaatcctcggtgaggtaattgcggaacaagaaggccaggaggtttatgaactggtcgaacaagcgcgcctgacttcttttgatatcgccaagggcaacgccgaaatggatagcctggttcaggttttcgacggcattactccagccaaggcaacaccgattgctcgcgcattttcccacttcgctctgctggctaacctggcggaagacctctacgatgaagagcttcgtgaacaggctctcgatgcaggcgacacccctccggacagcactcttgatgccacctggctgaaactcaatgagggcaatgttggcgcagaagctgtggccgatgtgctgcgcaatgctgaggtggcgccggttctgactgcgcacccaactgagactcgccgccgcactgtttttgatgcgcaaaagtggatcaccacccacatgcgtgaacgccacgctttgcagtctgcggagcctaccgctcgtacgcaaagcaagttggatgagatcgagaagaacatccgccgtcgcatcaccattttgtggcagaccgcgttgattcgtgtggcccgcccacgtatcgaggacgagatcgaagtagggctgcgctactacaagctgagccttttggaagagattccacgtatcaaccgtgatgtggctgttgagcttcgtgagcgtttcggcgagggtgttcctttgaagcccgtggtcaagccaggttcctggattggtggagaccacgacggtaacccttatgtcaccgcggaaacagttgagtattccactcaccgcgctgcggaaaccgtgctcaagtactatgcacgccagctgcattccctcgagcatgagctcagcctgtcggaccgcatgaataaggtcaccccgcagctgcttgcgctggcagatgcagggcacaacgacgtgccaagccgcgtggatgagccttatcgacgcgccgtccatggcgttcgcggacgtatcctcgcgacgacggccgagctgatcggcgaggacgccgttgagggcgtgtggttcaaggtctttactccatacgcatctccggaagaattcttaaacgatgcgttgaccattgatcattctctgcgtgaatccaaggacgttctcattgccgatgatcgtttgtctgtgctgatttctgccatcgagagctttggattcaacctttacgcactggatctgcgccaaaactccgaaagctacgaggacgtcctcaccgagcttttcgaacgcgcccaagtcaccgcaaactaccgcgagctgtctgaagcagagaagcttgaggtgctgctgaaggaactgcgcagccctcgtccgctgatcccgcacggttcagatgaatacagcgaggtcaccgaccgcgagctcggcatcttccgcaccgcgtcggaggctgttaagaaattcgggccacggatggtgcctcactgcatcatctccatggcatcatcggtcaccgatgtgctcgagccgatggtgttgctcaaggaattcggactcatcgcagccaacggcgacaacccacgcggcaccgtcgatgtcatcccactgttcgaaaccatcgaagatctccaggccggcgccggaatcctcgacgaactgtggaaaattgatctctaccgcaactacctcctgcagcgcgacaacgtccaggaagtcatgctcggttactccgattccaacaaggatggcggatatttctccgcaaactgggcgctttacgacgcggaactgcagctcgtcgaactatgccgatcagccggggtcaagcttcgcctgttccacggccgtggtggcaccgtcggccgcggtggcggaccttcctacgacgcgattcttgcccagcccaggggggctgtccaaggttccgtgcgcatcaccgagcagggcgagatcatctccgctaagtacggcaaccccgaaaccgcgcgccgaaacctcgaagccctggtctcagccacgcttgaggcatcgcttctcgacgtctccgaactcaccgatcaccaacgcgcgtacgacatcatgagtgagatctctgagctcagcttgaagaagtacgcctccttggtgcacgaggatcaaggcttcatcgattacttcacccagtccacgccgctgcaggagattggatccctcaacatcggatccaggccttcctcacgcaagcagacctcctcggtggaagatttgcgagccatcccatgggtgctcagctggtcacagtctcgtgtcatgctgccaggctggtttggtgtcggaaccgcattagagcagtggattggcgaaggggagcaggccacccaacgcattgccgagctgcaaacactcaatgagtcctggccatttttcacctcagtgttggataacatggctcaggtgatgtccaaggcagagctgcgtttggcaaagctctacgcagacctgatcccagatacggaagtagccgagcgagtctattccgtcatccgcgaggagtacttcctgaccaagaagatgttctgcgtaatcaccggctctgatgatctgcttgatgacaacccacttctcgcacgctctgtccagcgccgatacccctacctgcttccactcaacgtgatccaggtagagatgatgcgacgctaccgaaaaggcgaccaaagcgagcaagtgtcccgcaacattcagctgaccatgaacggtctttccactgcgctgcgcaactccggctag

SEQ ID NO: 6 - protein, 185 aa, Corynebacterium glutamicum
MNDQIHLDHQSDDTSECSCPIVVLVGLPGAGKSTIGRRLARALNTELVDSDELIERATGKACGAVFSELGEPAFRELEAIHVAEALKSSGVVSLGGGSVLTESTRELLKGQDVVWIDVPVEEGIRRTANERSRPVLQAADPAEHYRNLVKVRTPLYEEVATYRLRTNNRSPQQVVAAVLHHLEID

SEQ ID NO: 7 - protein, 174 aa, Escherichia coli
MTQPLFLIGPRGCGKTTVGMALADSLNRRFVDTDQWLQSQLNMTVAEIVEREEWAGFRARETAALEAVTAPSTVIATGGGIILTEFNRHFMQNNGIVVYLCAPVSVLVNRLQAAPEEDLRPTLTGKPLSEEVQEVLEERDALYREVAHIIIDATNEPSQVISEIRSALAQTINC

SEQ ID NO: 8 - DNA, 179 bp, artificial sequence
  Pomotorsequenz
cacagggtagctggtagtttgaaaatcaacgccgttgcccttaggattcagtaactggcacattttgtaatgcgctagatctgtgtgctcagtcttccaggctgcttatcacagtgaaagcaaaaccaattcgtggctgcgaaagtcgtagccaccacgaagtccaggaggacatacat

SEQ ID NO: 9 - protein, 430 aa, Escherichia coli
MVFVSDSSISLPIWDAPRARGPIVSDLAIPGSKSITNRALILAALASTPSTIIDVLRSRDTDLMTDGLRSLGITITEEAVDRYRVEPGQLSAGSVECGLAGTVMRFLPPVAAFADGPVHFDGDPQARVRPMTSILDALRSLGVEVDNNNLPFTVNAGEVPEGGVVEIDASGSSQFVSGLLLSAPRFKNGVTVKHVGGRLPSMPHIEMTVDMLRSAGIEIEESENQWVVHPGEILGRTWRIEPDLSNATPFLAAAAVTGGTIKINHWPIKTTQPGDAIRSILERMGCEVELVAQGEGYDLSVTGPVALKGIEIDMSDIGELTPTVAALAALASTESRLTGIAHLRGHETDRLAALTAEINKLGGKCTELKDGLLIEPASLHGGVWHSYADHRMATAGAIIGLAVDGVQVEDIKTTSKTFPGFENVWEEMVG

SEQ ID NO: 10 - protein, 410 aa, Corynebacterium glutamicum
MLGMLRWTTAGESHGQALIATVEHMPAGVPVTKDEVSYQLARRRLGYGRGARMKFEQDALTFLTGIRHGLTLGSPISIMIGNTEWDKWTTIMSSDALDMEDPDNVAAMSSGRGAKLTRPRPGHADYAGMLKYGFDDARNVLERSSARETAARVAAATVARSFLRETLGVEVLSHVISIGASEPYTGAEPTFADIQAIDDSPVRAFGKDAEESMIAEIEAAKKAGDTLGGIVEVIVEGLPIGLGSHISGEDRLDAQIAAALMGIQAIKGVEIGDGFEEARRRGSEAHDEVFLDDNGVYRNTNRAGGLEGGMTNGETLRVRAGMKPISTVPRALKTIDMENGKAATGIHQRSDVCAVPAAGVVAEAMVTLVLARAVLQKFGGDSLSETKSNIDTYLKNIEERMKFEGLEDGA

SEQ ID NO: 11 - protein, 350 aa, artificial sequence
  modifiziertes Enzym
MNYQNDDLRIKEIKELLPPVALLEKFPATENAANTVAHARKAIHKILKGNDDRLLVVIGPCSIHDPVAAKEYATRVLALREELKDELEIVMRVYFEKPRTTVGWKGLINDPHMDNSFQINDGLRIARKLLLDINDSGLPAAGEFLDMITPQYLADLMSWGAIGARTTESQVHRELASGLSCPVGFKNGTDGTIKVAIDAINAAGAPHCFLFVTKWGHSAIVNTSGNGDCHIILRGGKEPNYSAKHVAEVKEGLNKAGLPAQVMIDFSHANSSKQFKKQMDVCADVCQQIAGGEKAIIGVMVESHLVEGNQSLESGEPLAYGKSITDACIGWEDTDALLRQLANAVKARRG

SEQ ID NO: 12 - protein, 446 aa, Xanthomonas campestris
MSNTVFIGAKEYFPGIGKIGFEGRDSDNPLAFKVYDANKQVAGKTMAEHLRFAVAYWHSFCGNGADPFGPGTRAYPWDVGNTALARAEAKSDAAFEFFTKLGVPYYCFHDIDLAPDADDIGEYENNLKHMVGIAKQRQADTGVKLLWGTANLFSHPRYMNGASTNPDFNVVARAAVQVKAAIDATVELGGENYVFWGGREGYACLHNTQMKREQDNMARFLTLARDYGRAIGFTGNFLIEPKPMEPMKHQYDFDSATVIGFLRQHGLDQDFKLNIEANHATLSGHSFEHDLQVASDAGLLGSIDANRGNPQNGWDTDQFPTDLYDTVGAMLVVLRQGGLAPGGLNFDAKVRRESSDPQDLFLAHIGGMDAFARGLEVANALLTSSPLETWRAQRYASFDSGAGADFANGTSTLADLAKYAAGKGEPTQVSGRQEAYENLINQYLTR

SEQ ID NO: 13 - protein, 463 aa, artificial sequence
  modifiziertes Enzym
MSNTVFIGAKEYFPGIGKIGFEGRDSDNPLAFKVYDANKQVAGKTMAEHLRFAVAYWHSFCGNGADPFGPGTRAYPWDVGNTALARAEAKSDAAFEFFTKLGVPYYCFHDIDLAPDADDIGEYENNLKHMVGIAKQRQADTGVKLLWGTANLFSHPRYMNGASTNPDFNVVARAAVQVKAAIDATVELGGENYVFWGGREGYACLHNTQMKREQDNMARFLTLARDYGRAIGFTGNFLIEPKPMEPMKHQYDFDSATVIGFLRQHGLDQDFKLNIEANHATLSGHSFEHDLQVASDAGLLGSIDANRGNPQNGWDTDQFPTDLYDTVGAMLVVLRQGGLAPGGLNFDAKVRRESSDPQDLFLAHIGGMDAFARGLEVANALLTSSPLETWRAQRYASFDSGAGADFANGTSTLADLAKYAAGKGEPTQVSGRQEAYENLINQYLTRHRVAGSLKINAVALRIQ

SEQ ID NO: 14 - protein, 460 aa, Corynebacterium glutamicum
MALVLGIDSSTQSCKALLVDAATGQVIDEGRASHPSGSEVDPRAWIAALDQATEGLLERADAVSIAGQQHGMVALDENDEIVRPALLWNDTRSAQAALDLNEEIGGDQAAVDATGSVYVASLTATKMRWMRDHEPENAARTASVMLPHDFLTWHLMGRGRKVTDHGDASGTGYYSTRDRAWRTDLAALALGHEVELPELLAPNAIAGTTPGGVKVAAGTGDNAAAALGLDLQPGDVSVSIGTSGVAGMTVQHSVHDPSGLVTGFADATGAYFPLACTLNGAPVLEFGRRILGVEWEEFDALALAAQPGSGGVTLQPYLEGERTPNRPAARGVLAGLNCATTREDFARATVEGLLLALDDAVTALVEATGVPVQRIQLIGGGARSQAVREIAPEIFGHEIVVPEPAEYVALGAARQAAWALSGEATPPQWPTPGSDPHRAPKNTELSTRYAKLRAATQGWY

SEQ ID NO: 15 - DNA, 3302 bp, artificial sequence
  Expressionskonstrukt
gatcccacagggtagctggtagtttgaaaatcaacgccgttgcccttaggattcagtaactggcacattttgtaatgcgctagatctgtgtgctcagtcttccaggctgcttatcacagtgaaagcaaaaccaattcgtggctgcgaaagtcgtagccaccacgaagtccaggaggacatacagtatgacacaacctctttttctgatcgggcctcggggctgtggtaaaacaacggtcggaatggcccttgccgattcgcttaaccgtcggtttgtcgataccgatcagtggttgcaatcacagctcaatatgacggtcgcggagatcgtcgaaagggaagagtgggcgggatttcgcgccagagaaacggcggcgctggaagcggtaactgcgccatccaccgttatcgctacaggcggcggcattattctgacggaatttaatcgtcacttcatgcaaaataacgggatcgtggtttatttgtgtgcgccagtatcagtcctggttaaccgactgcaagctgcaccggaagaagatttacggccaaccttaacgggaaaaccgctgagcgaagaagttcaggaagtgctggaagaacgcgatgcgctatatcgcgaagttgcgcatattatcatcgacgcaacaaacgaacccagccaggtgatttctgaaattcgcagcgccctggcacagacgatcaattgttgacaatctttagaggagacacaacatggtctttgtgtctgattcgtctatctctttgcccatttgggatgctccgcgcgctcgcggccccatagtctcggacctggctatccctggttccaagtcgatcaccaaccgcgccctcatcttggctgcgctcgcatcaactccatccaccatcattgatgtccttcgtagtcgtgataccgatctcatgactgatggtctacgcagcctcggaatcaccattactgaagaggcagtcgatcgctaccgcgttgagcccggacagttgtctgctggctccgttgagtgtggtcttgctggtacggtcatgcgctttttgcctcctgttgctgctttcgctgatggtcctgttcattttgatggcgatcctcaagctcgtgttcgtccgatgaccagcattttggatgcgctgcgttcgcttggtgtggaggtagacaacaacaatctgcctttcactgttaatgctggtgaggtccctgagggtggcgtggttgagattgatgcttccggctcatctcagtttgtttctggtcttttgctttcagcgcctcgttttaaaaatggcgtcaccgttaagcacgtcggtggtcgtctgccgagcatgccgcatattgagatgaccgtcgatatgcttcgttccgcaggcattgagatcgaagagtcagaaaatcagtgggttgttcatcctggtgagatcttgggtcggacctggcgcattgagccggatctttctaatgcgactccgttcctagctgccgctgcggtcactggtggaaccatcaagattaaccactggccaatcaaaactactcagcctggcgatgctattcgttcgattcttgagcgcatgggctgcgaagttgagctggttgctcagggtgaaggttacgatctgtcggtgactggtccggttgctctcaagggcattgagatcgatatgtccgatatcggtgagttgacccctaccgtggcggcgttggctgcgttggcgtcgacagagtctcgtttgaccggtattgctcatcttcgtggccatgagacggatcgtttggctgcgttgactgcggagatcaacaaacttggtggaaagtgcactgagcttaaggatggtctgttgattgagcctgcgtcgctgcacggtggtgtgtggcattcatatgctgatcaccgtatggctactgctggtgcgatcattggcctcgcggttgatggcgttcaggttgaagacattaagaccacttccaaaactttccctggttttgaaaatgtttgggaggagatggttggctaggcgaaagtcgtagccaccacgaagtccgaaaggaggcccttcagatgctaggcatgcttcgatggactacagcaggtgaatcccacggccaggcgcttatcgccacggttgaacacatgccagcaggcgtgcccgtgactaaagatgaggtctcgtatcaattggcgcgccgacgccttggatatggtcgcggcgctcgcatgaagtttgagcaagacgcgttgaccttcctcaccggcatccgccacggcctcactttgggtagccccatctcaatcatgatcggcaacactgagtgggataagtggaccaccatcatgtcctctgacgctttggacatggaagacccagataacgttgcggcgatgtcttcgggtcggggcgcaaaactgactcgtccgcgtccaggccacgctgattacgcaggcatgctcaagtacggattcgatgatgcccgcaacgtgctggagcgttcttcagcccgtgagacggcagcacgcgtggcagcagcaaccgttgcgcgttccttcctgcgtgaaaccttgggcgtggaagtgctttcccacgtaatttccattggtgcgtccgagccttacactggcgcggagccaacctttgcagatattcaagcaatcgatgattccccagttcgtgcattcggtaaagacgctgaagaatccatgatcgcggaaatcgaggccgcaaagaaagccggcgataccctcggtggcatcgtggaagtgattgttgaaggcctgcccatcggtttgggctcacacatttctggcgaagatcgcctcgatgcgcagatcgcagctgcactcatgggcattcaggccatcaagggcgtggaaatcggtgacggtttcgaagaagctcgtcgacgtggctccgaagcccacgatgaagtgttcctggatgacaacggcgtataccgcaacaccaaccgtgcaggtggcctcgaaggcggcatgaccaacggtgaaaccctgcgcgttcgtgctggcatgaagccaatttctactgtgcctcgcgccctgaaaaccattgatatggaaaacggcaaggcagcaaccggaatccaccagcgttccgacgtgtgcgctgttccagccgccggtgtcgttgcagaagcaatggtcaccctggttctcgcccgcgcagtcctgcagaaattcggcggtgactccctgagcgaaaccaagagcaacattgacacctacctcaaaaacattgaggaacgaatgaaattcgaaggtttagaggatggagcgtaa

SEQ ID NO: 16 - DNA, 3539 bp, artificial sequence
  Expressionskonstrukt
cacagggtagctggtagtttgaaaatcaacgccgttgcccttaggattcagtaactggcacattttgtaatgcgctagatctgtgtgctcagtcttccaggctgcttatcacagtgaaagcaaaaccaattcgtggctgcgaaagtcgtagccaccacgaagtccaggaggacatacatgaaaggaggcccttcagatgtccaacaccgtgttcatcggcgcaaaggaatacttcccaggcatcggcaagatcggcttcgaaggccgcgattccgataacccactggcattcaaggtgtacgatgcaaacaagcaggtggcaggcaagaccatggcagaacacctgcgcttcgcagtggcatactggcactccttctgcggcaacggcgcagatccattcggcccaggcacccgcgcatacccatgggatgtgggcaacaccgcactggcacgcgcagaagcaaagtccgatgcagcattcgaattcttcaccaagctgggcgtgccatactactgcttccacgatatcgatctggcaccagatgcagatgatatcggcgaatacgaaaacaacctgaagcacatggtgggcatcgcaaagcagcgccaggcagataccggcgtgaagctgctgtggggcaccgcaaacctgttctcccacccacgctacatgaacggcgcatccaccaacccagatttcaacgtggtggcacgcgcagcagtgcaggtgaaggcagcaatcgatgcaaccgtggaactgggcggcgaaaactacgtgttctggggcggccgcgaaggctacgcatgcctgcacaacacccagatgaagcgcgaacaggataacatggcacgcttcctgaccctggcacgcgattacggccgcgcaatcggcttcaccggcaacttcctgatcgaaccaaagccaatggaaccaatgaagcaccagtacgatttcgattccgcaaccgtgatcggcttcctgcgccagcacggcctggatcaggatttcaagctgaacatcgaagcaaaccacgcaaccctgtccggccactccttcgaacacgatctgcaggtggcatccgatgcaggcctgctgggctccatcgatgcaaaccgcggcaacccacagaacggctgggataccgatcagttcccaaccgatctgtacgataccgtgggcgcaatgctggtggtgctgcgccagggcggcctggcaccaggcggcctgaacttcgatgcaaaggtgcgccgcgaatcctccgatccacaggatctgttcctggcacacatcggcggcatggatgcattcgcacgcggcctggaagtggcaaacgcactgctgacctcctccccactggaaacctggcgcgcacagcgctacgcatccttcgattccggcgcaggcgcagatttcgcaaacggcacctccaccctggcagatctggcaaagtacgcagcaggcaagggcgaaccaacccaggtgtccggccgccaggaagcatacgaaaacctgatcaaccagtacctgacccgccacagggtagctggtagtttgaaaatcaacgccgttgcccttaggattcagtaactggcacattttgtaatgcgctagatctgtgtgctcagtcttccaggctgcttatcacagtgaaagcaaaaccaattcgtggctgcgaaagtcgtagccaccacgaagtccaggaggacatacatgaaaggaggcccttcagatggctttggttcttggaatcgatagttccacccaatcctgcaaggctttgcttgtcgatgccgccaccggccaggttatcgacgaaggccgcgcgagtcacccgagcgggtcggaggtagatccacgtgcgtggatcgctgcgctggatcaagctaccgaggggttgttagaacgcgcggacgctgtatctattgcaggccagcagcacggcatggtggcgttggatgaaaacgatgaaatcgttcgcccggcgttgttatggaatgacactcgttctgcccaggctgcgttggatctcaatgaggagatcggcggcgatcaggctgcggtagatgccacgggaagtgtgtatgttgcttctttaactgccaccaaaatgcggtggatgcgtgatcatgaaccagaaaatgcagcgcgcacggcgtcggtgatgttgcctcatgatttcctcacctggcatttgatgggacgcggacgcaaagtcaccgaccatggtgatgcttctggaacgggctactacagcacgcgtgatcgtgcgtggcgcaccgatctagctgccttggcgctgggccatgaggtggaacttcctgaactcctggccccaaatgcgattgcgggaacaactccaggtggagtgaaagttgctgcaggcacgggagataatgctgcggctgcgcttggccttgatttgcagcctggtgatgtcagcgtgtcgatcggcacctctggcgttgccggcatgaccgttcaacatagcgtccacgatccatctggtttggtcactggtttcgccgatgccacgggtgcgtatttcccgctggcctgcacgcttaatggcgcaccggtgttggaattcggccgccgcattctgggcgtggaatgggaagagttcgatgcgcttgcactggctgctcaacccggttcaggtggcgtgacgctccagccttatttggagggcgagcgtacgccgaatcgtcccgcagcacgtggcgttttggctggactaaactgtgcaacgacccgcgaggactttgcccgagcaactgttgaaggcttgttgttggcattggatgatgctgtaacggcgctggttgaggccacgggagtgcccgttcagcgcatccagctcatcggtggcggcgcgcgttcacaggcggttcgtgagattgcccctgagattttcggccatgagattgtggttccagaacccgctgaatatgtggcgttgggtgcagctcgtcaggcggcatgggcgctgtcgggtgaggccacgccaccgcagtggccaactcccggttccgatccgcaccgcgcacctaaaaacactgagctgagcacgcgttatgcgaagctgcgtgctgcaacgcagggttggtactagggctgttttggcggatgagagaagattttcagcctgatacagattaaatcagaacgcagaagcggtctgataaaacagaatttgcctggcggcagtagcgcggtggtcccacctgaccccatgccgaactcagaagtgaaacgccgtagcgccgatggtagtgtggggtctccccatgcgagagtagggaactgccaggcatcaaataaaacgaaaggctcagtcgaaagactgggcctttcgttttatctgttgtttgtcggtgaacgctctcctgagtaggacaaatccgccgggagcggatttgaacgttgcgaagcaacggcccggagggtggcgggcaggacgcccgccataaactgccaggcatcaaattaagcagaaggccatcctgacggatggcctttttgcgtttctacaaactct

SEQ ID NO: 17 - DNA, 1101 bp, Corynebacterium glutamicum
atgagttctccagtctcactcgaaaacgcggcgtcaaccagcaacaagcgcgtcgtggctttccacgagctgcctagccctacagatctcatcgccgcaaacccactgacaccaaagcaggcttccaaggtggagcaggatcgccaggacatcgctgatatcttcgctggcgacgatgaccgcctcgttgtcgttgtgggaccttgctcagttcacgatcctgaagcagccatcgattacgcaaaccgcctggctccgctggcaaagcgccttgatcaggacctcaagattgtcatgcgcgtgtacttcgagaagcctcgcaccatcgtcggatggaagggattgatcaatgatcctcacctcaacgaaacctacgacatcccagagggcttgcgcattgcgcgcaaagtgcttatcgacgttgtgaaccttgatctcccagtcggctgcgaattcctcgaaccaaacagccctcagtactacgccgacactgtcgcatggggagcaatcggcgctcgtaccaccgaatctcaggtgcaccgccagctggcttctgggatgtctatgccaattggtttcaagaacggaactgacggaaacatccaggttgcagtcgacgcggtacaggctgcccagaacccacacttcttcttcggaacctccgacgacggcgcgctgagcgtcgtggagaccgcaggcaacagcaactcccacatcattttgcgcggcggtacctccggcccgaatcatgatgcagcttcggtggaggccgtcgtcgagaagcttggtgaaaacgctcgtctcatgatcgatgcttcccatgctaactccggcaaggatcatatccgacaggttgaggttgttcgtgaaatcgcagagcagatttctggcggttctgaagctgtggctggaatcatgattgagtccttcctcgttggtggcgcacagaaccttgatcctgcgaaattgcgcatcaatggcggtgaaggcctggtgtacggacagtctgtgaccgataagtgcatcgatattgacaccaccatcgatttgctcgctgagctggccgcagcagtaagggaacgccgagcagcagccaagtaa

SEQ ID NO: 18 - protein, 366 aa, artificial sequence
  Modifiziertes Enzym
MSSPVSLENAASTSNKRVVAFHELPSPTDLIAANPLTPKQASKVEQDRQDIADIFAGDDDRLVVVVGPCSVHDPEAAIDYANRLAPLAKRLDQDLKIVMRVYFEKPRTIVGWKGLINDPHLNETYDIPEGLRIARKVLIDVVNLDLPVGCEFLNPNSPQYYADTVAWGAIGARTTESQVHRQLASGMSMPIGFKNGTDGNIQVAVDAVQAAQNPHFFFGTSDDGALSVVETAGNSNSHIILRGGTSGPNHDAASVEAVVEKLGENARLMIDASHANSGKDHIRQVEVVREIAEQISGGSEAVAGIMIESFLVGGAQNLDPAKLRINGGEGLVYGQSVTDKCIDIDTTIDLLAELAAAVRERRAAAK